European Patent Application EP 4 567 117 A2, published June 11, 2025. Title: ENGINEERED MAD7 DIRECTED ENDONUCLEASE. Applicant: BIO-TECHNE CORPORATION. Application EP. The sequence listing filed with the application follows.

SEQUENCE LISTING (344 sequences)

SEQ ID NO: 1 - protein, 1263 aa, Eubacterium rectale
MNNGTNNFQNFIGISSLQKTLRNALIPTETTQQFIVKNGIIKEDELRGENRQILKDIMDDYYRGFISETLSSIDDIDWTSLFEKMEIQLKNGDNKDTLIKEQTEYRKAIHKKFANDDRFKNMFSAKLISDILPEFVIHNNNYSASEKEEKTQVIKLFSRFATSFKDYFKNRANCFSADDISSSSCHRIVNDNAEIFFSNALVYRRIVKSLSNDDINKISGDMKDSLKEMSLEEIYSYEKYGEFITQEGISFYNDICGKVNSFMNLYCQKNKENKNLYKLQKLHKQILCIADTSYEVPYKFESDEEVYQSVNGFLDNISSKHIVERLRKIGDNYNGYNLDKIYIVSKFYESVSQKTYRDWETINTALEIHYNNILPGNGKSKADKVKKAVKNDLQKSITEINELVSNYKLCSDDNIKAETYIHEISHILNNFEAQELKYNPEIHLVESELKASELKNVLDVIMNAFHWCSVFMTEELVDKDNNFYAELEEIYDEIYPVISLYNLVRNYVTQKPYSTKKIKLNFGIPTLADGWSKSKEYSNNAIILMRDNLYYLGIFNAKNKPDKKIIEGNTSENKGDYKKMIYNLLPGPNKMIPKVFLSSKTGVETYKPSAYILEGYKQNKHIKSSKDFDITFCHDLIDYFKNCIAIHPEWKNFGFDFSDTSTYEDISGFYREVELQGYKIDWTYISEKDIDLLQEKGQLYLFQIYNKDFSKKSTGNDNLHTMYLKNLFSEENLKDIVLKLNGEAEIFFRKSSIKNPIIHKKGSILVNRTYEAEEKDQFGNIQIVRKNIPENIYQELYKYFNDKSDKELSDEAAKLKNVVGHHEAATNIVKDYRYTYDKYFLHMPITINFKANKTGFINDRILQYIAKEKDLHVIGIDRGERNLIYVSVIDTCGNIVEQKSFNIVNGYDYQIKLKQQEGARQIARKEWKEIGKIKEIKEGYLSLVIHEISKMVIKYNAIIAMEDLSYGFKKGRFKVERQVYQKFETMLINKLNYLVFKDISITENGGLLKGYQLTYIPDKLKNVGHQCGCIFYVPAAYTSKIDPTTGFVNIFKFKDLTVDAKREFIKKFDSIRYDSEKNLFCFTFDYNNFITQNTVMSKSSWSVYTYGVRIKRRFVNGRFSNESDTIDITKDMEKTLEMTDINWRDGHDLRQDIIDYEIVQHIFEIFRLTVQMRNSLSELEDRDYDRLISPVLNENNIFYDSAKAGDALPKDADANGAYCIALKGLYEIKQITENWKEDGKFSRDKLKISNKDWFDFIQNKRYL

SEQ ID NO: 2 - protein, 179 aa, Eubacterium rectale
PAAYTSKIDPTTGFVNIFKFKDLTVDAKREFIKKFDSIRYDSEKNLFCFTFDYNNFITQNTVMSKSSWSVYTYGVRIKRRFVNGRFSNESDTIDITKDMEKTLEMTDINWRDGHDLRQDIIDYEIVQHIFEIFRLTVQMRNSLSELEDRDYDRLISPVLNENNIFYDSAKAGDALPKDA

SEQ ID NO: 3 - protein, 56 aa, synthetic construct
  REGION 1..56: note = Synthetic
KTGFINDRILQYIAKEKDLHVIGIDRGERNLIYVSVIDTCGNIVEQKSFNIVNGYD

SEQ ID NO: 4 - protein, 108 aa, synthetic construct
  REGION 1..108: note = Synthetic
EWKEIGKIKEIKEGYLSLVIHEISKMVIKYNAIIAMEDLSYGFKKGRFKVERQVYQKFETMLINKLNYLVFKDISITENGGLLKGYQLTYIPDKLKNVGHQCGCIFYV

SEQ ID NO: 5 - protein, 51 aa, synthetic construct
  REGION 1..51: note = Synthetic
DANGAYCIALKGLYEIKQITENWKEDGKFSRDKLKISNKDWFDFIQNKRYL

SEQ ID NO: 6 - protein, 93 aa, synthetic construct
  REGION 1..93: note = Synthetic
LPGPNKMIPKVFLSSKTGVETYKPSAYILEGYKQNKHIKSSKDFDITFCHDLIDYFKNCIAIHPEWKNFGFDFSDTSTYEDISGFYREVELQG

SEQ ID NO: 7 - protein, 84 aa, synthetic construct
  REGION 1..84: note = Synthetic
MTNLSDIIEKETGKQLVIQESILMLPEEVEEVIGNKPESDILVHTAYDESTDENVMLLTSDAPEYKPWALVIQDSNGENKIKML

SEQ ID NO: 8 - protein, 219 aa, synthetic construct
  REGION 1..219: note = Synthetic
KGHLTRLGLEFFDQPAVPLARAFLGQVLVRRLPNGTELRGRIVETQAYLGPEDEAAHSRGGRQTPRNRGMFMKPGTLYVYIIYGMYFCMNISSQGDGACVLLRALEPLEGLETMRQLRSTLRKGTASRVLKDRELCSGPSKLCQALAINKSFDQRDLAQDEAVWLERGPLEPSEPAVVAAARVGVGHAGEWARKPLRFYVRGSPWVSVVDRVAEQDTQA

SEQ ID NO: 9 - protein, 222 aa, synthetic construct
  REGION 1..222: note = Synthetic
DLASLRAQQIELASSVIREDRLDKDPPDLIAGAAVGFEQGGEVTRAAMVLLKYPSLELVEYKVARIATTMPYIPGFLSFREYPALLAAWEMLSQKPDLVFVDGHGISHPRRLGVASHFGLLVDVPTIGVAKKRLCGKFEPLSSEPGALAPLMDKGEQLAWVWRSKARCNPLFIATGHRVSVDSALAWVQRCMKGYRLPEPTRWADAVASERPAFVRYTANQP

SEQ ID NO: 10 - protein, 636 aa, synthetic construct
  REGION 1..636: note = Synthetic
MMLNWLKSGKLESQSQEQSSCYLENSNCLPPILDSTDIIGEENKAGITSRKKRKYDEDYLNFGFTWIGDKDEPNGLCVICEQVVNNSSLNPAKLKRHLDTKHPILKGKSEYFKRKCNELNQKKHTFERYVRDDNKNLLKASYLVSLRIAKQGEAYTIAEKLIKPCIKDLITCVFGEKFASKVDLVPLSDITISRRIEDMSYFCEAVLVNRLKNAKCGFTLQMDESTDVAGLAILLVFVRYIHESSFEEDMLFCKALPTQTTGEEIFNLLNAYFEKHSIPWNLCYHICIDGAKAMVGVIKGVIARIKKLVPDIKASHCCLHRHALAVKRIPNALHEVLNDAVKMINFIKSRPLNARVFALLCDDLGSLHKNLLLHTEVRWLSRGKVLTRFWELRDEIRIFFNEREFAGKLNDTSWLQNLAYIADIFSYLNEVNLSLQGPNSTIFKVNSRINSIKSKLKLWEECITKNNTECFANLNDFLETSNTALDPNLKSNILEHLNGLKNIFLEYFPPTCNNISWVENPFNECGNVDTLPIKEREQLIDIRIDTTLKSSFVPDGIGPFWIKLMDEFFEISKRAVKELMPFVTTYLCEKSFSVYVATKTKYRNRLDAEDDMRLQLTTIHPDIDNLCNNKQAQKSH

SEQ ID NO: 11 - protein, 4 aa, synthetic construct
  REGION 1..4: note = Synthetic
YTTV

SEQ ID NO: 12 - protein, 4 aa, synthetic construct
  REGION 1..4: note = Synthetic
TTTN

SEQ ID NO: 13 - protein, 4 aa, synthetic construct
  REGION 1..4: note = Synthetic
CTTN

SEQ ID NO: 14 - DNA, 21 bp, synthetic construct
  misc_feature 1..21: note = Synthetic
  source 1..21: mol_type = other DNA
ttaatttctactcttgtagat

SEQ ID NO: 15 - protein, 9 aa, synthetic construct
  REGION 1..9: note = Synthetic
GSGGSGGSG

SEQ ID NO: 16 - protein, 12 aa, synthetic construct
  REGION 1..12: note = Synthetic
GSGGSGGSGGSG

SEQ ID NO: 17 - protein, 10 aa, synthetic construct
  REGION 1..10: note = Synthetic
GGGGGGGGGG

SEQ ID NO: 18 - protein, 14 aa, synthetic construct
  REGION 1..14: note = Synthetic
KLGGGAPAVGGGPK

SEQ ID NO: 19 - protein, 15 aa, synthetic construct
  REGION 1..15: note = Synthetic
GGSGGSGGSGGSGTS

SEQ ID NO: 20 - protein, 18 aa, synthetic construct
  REGION 1..18: note = Synthetic
KLGGGAPAVGGGPKAADK

SEQ ID NO: 21 - protein, 19 aa, synthetic construct
  REGION 1..19: note = Synthetic
EFGGGGSGGGGSGGGGSQF

SEQ ID NO: 22 - protein, 10 aa, synthetic construct
  REGION 1..10: note = Synthetic
SGGSGGSGGS

SEQ ID NO: 23 - RNA, 41 nt, synthetic construct
  misc_feature 1..41: note = Synthetic
  source 1..41: mol_type = other RNA
taatttctactcttgtagatccgtcaccaaaatcagattca

SEQ ID NO: 24 - DNA, 4147 bp, Cloning vector pTrichoGate-19
  source 1..4147: mol_type = unassigned DNA
agccacttccaattacaaagcacagtatgtatacttcaaacttaagtggtgaacttaggctccgctccttatgggttttctaatgttaatttttagaatctgggtccattagctgtttagagcaaatattgttatcctgtagtccaaggagggtatagataagcatgttttccaagaaaagggtctggagctttcattagattctcataggatttttaccgtcaccaaaatcagattcagaaccacttctctaaaaatatggctctattctctctcccatcctcaggttagcttcttgtaccttccctcccctagcaacgcccctttaaagaagctaagttggaaatggtctctttcctcaggtgtattttgacctacgaattggagatgaagatgtaggccgggtgatctttggtctcttcggaaagactgttccaaaaacagtggataattttgtggccttagctacaggagaggtaagtggctggagcaggggtagtcaactcacatgaagtgaaattggcactggggatggcagcaaactgacctgcagagttcagccgatctgtagcgtggacctcactgagcaccgactgcctgttgccctgggaacacagtattgccctttaagggcgaattctgcagatatccatcacactggcggccgctcgagcatgcatctagagggcccaattcgccctatagtgagtcgtattacaattcactggccgtcgttttacaacgtcgtgactgggaaaaccctggcgttacccaacttaatcgccttgcagcacatccccctttcgccagctggcgtaatagcgaagaggcccgcaccgatcgcccttcccaacagttgcgcagcctatacgtacggcagtttaaggtttacacctataaaagagagagccgttatcgtctgtttgtggatgtacagagtgatattattgacacgccggggcgacggatggtgatccccctggccagtgcacgtctgctgtcagataaagtctcccgtgaactttacccggtggtgcatatcggggatgaaagctggcgcatgatgaccaccgatatggccagtgtgccggtctccgttatcggggaagaagtggctgatctcagccaccgcgaaaatgacatcaaaaacgccattaacctgatgttctggggaatataaatgtcaggcatgagattatcaaaaaggatcttcacctagatccttttcacgtagaaagccagtccgcagaaacggtgctgaccccggatgaatgtcagctactgggctatctggacaagggaaaacgcaagcgcaaagagaaagcaggtagcttgcagtgggcttacatggcgatagctagactgggcggttttatggacagcaagcgaaccggaattgccagctggggcgccctctggtaaggttgggaagccctgcaaagtaaactggatggctttctcgccgccaaggatctgatggcgcaggggatcaagctctgatcaagagacaggatgaggatcgtttcgcatgattgaacaagatggattgcacgcaggttctccggccgcttgggtggagaggctattcggctatgactgggcacaacagacaatcggctgctctgatgccgccgtgttccggctgtcagcgcaggggcgcccggttctttttgtcaagaccgacctgtccggtgccctgaatgaactgcaagacgaggcagcgcggctatcgtggctggccacgacgggcgttccttgcgcagctgtgctcgacgttgtcactgaagcgggaagggactggctgctattgggcgaagtgccggggcaggatctcctgtcatctcaccttgctcctgccgagaaagtatccatcatggctgatgcaatgcggcggctgcatacgcttgatccggctacctgcccattcgaccaccaagcgaaacatcgcatcgagcgagcacgtactcggatggaagccggtcttgtcgatcaggatgatctggacgaagagcatcaggggctcgcgccagccgaactgttcgccaggctcaaggcgagcatgcccgacggcgaggatctcgtcgtgacccatggcgatgcctgcttgccgaatatcatggtggaaaatggccgcttttctggattcatcgactgtggccggctgggtgtggcggaccgctatcaggacatagcgttggctacccgtgatattgctgaagagcttggcggcgaatgggctgaccgcttcctcgtgctttacggtatcgccgctcccgattcgcagcgcatcgccttctatcgccttcttgacgagttcttctgaattattaacgcttacaatttcctgatgcggtattttctccttacgcatctgtgcggtatttcacaccgcatacaggtggcacttttcggggaaatgtgcgcggaacccctatttgtttatttttctaaatacattcaaatatgtatccgctcatgagacaataaccctgataaatgcttcaataatagcacgtgaggagggccaccatggccaagttgaccagtgccgttccggtgctcaccgcgcgcgacgtcgccggagcggtcgagttctggaccgaccggctcgggttctcccgggacttcgtggaggacgacttcgccggtgtggtccgggacgacgtgaccctgttcatcagcgcggtccaggaccaggtggtgccggacaacaccctggcctgggtgtgggtgcgcggcctggacgagctgtacgccgagtggtcggaggtcgtgtccacgaacttccgggacgcctccgggccggccatgaccgagatcggcgagcagccgtgggggcgggagttcgccctgcgcgacccggccggcaactgcgtgcacttcgtggccgaggagcaggactgacacgtgctaaaacttcatttttaatttaaaaggatctaggtgaagatcctttttgataatctcatgaccaaaatcccttaacgtgagttttcgttccactgagcgtcagaccccgtagaaaagatcaaaggatcttcttgagatcctttttttctgcgcgtaatctgctgcttgcaaacaaaaaaaccaccgctaccagcggtggtttgtttgccggatcaagagctaccaactctttttccgaaggtaactggcttcagcagagcgcagataccaaatactgtccttctagtgtagccgtagttaggccaccacttcaagaactctgtagcaccgcctacatacctcgctctgctaatcctgttaccagtggctgctgccagtggcgataagtcgtgtcttaccgggttggactcaagacgatagttaccggataaggcgcagcggtcgggctgaacggggggttcgtgcacacagcccagcttggagcgaacgacctacaccgaactgagatacctacagcgtgagctatgagaaagcgccacgcttcccgaagggagaaaggcggacaggtatccggtaagcggcagggtcggaacaggagagcgcacgagggagcttccagggggaaacgcctggtatctttatagtcctgtcgggtttcgccacctctgacttgagcgtcgatttttgtgatgctcgtcaggggggcggagcctatggaaaaacgccagcaacgcggcctttttacggttcctgggcttttgctggccttttgctcacatgttctttcctgcgttatcccctgattctgtggataaccgtattaccgcctttgagtgagctgataccgctcgccgcagccgaacgaccgagcgcagcgagtcagtgagcgaggaagcggaagagcgcccaatacgcaaaccgcctctccccgcgcgttggccgattcattaatgcagctggcacgacaggtttcccgactggaaagcgggcagtgagcgcaacgcaattaatgtgagttagctcactcattaggcaccccaggctttacactttatgcttccggctcgtatgttgtgtggaattgtgagcggataacaatttcacacaggaaacagctatgaccatgattacgccaagctatttaggtgacactatagaatactcaagctatgcatcaagcttggtaccgagctcggatccactagtaacggccgccagtgtgctggaattcgccctt

SEQ ID NO: 25 - DNA, 57 bp, synthetic construct
  misc_feature 1..57: note = Synthetic
  source 1..57: mol_type = other DNA
tttagagaagtggttctgaatctgattttggtgacggtaaaaatcctatgagaatct

SEQ ID NO: 26 - DNA, 57 bp, synthetic construct
  misc_feature 1..57: note = Synthetic
  source 1..57: mol_type = other DNA
agattctcataggatttttaccgtcaccaaaatcagattcagaaccacttctctaaa

SEQ ID NO: 27 - DNA, 23 bp, synthetic construct
  misc_feature 1..23: note = Synthetic
  source 1..23: mol_type = other DNA
agtgggggtgaattcagtgtagt

SEQ ID NO: 28 - DNA, 20 bp, synthetic construct
  misc_feature 1..20: note = Synthetic
  source 1..20: mol_type = other DNA
gtcaccaatcctgtccctat

SEQ ID NO: 29 - protein, 27 aa, synthetic construct
  REGION 1..27: note = Synthetic
FSADDISSSSCHRIVNDNAEIFFSNAL

SEQ ID NO: 30 - protein, 27 aa, synthetic construct
  REGION 1..27: note = Synthetic
YSSNDIPTSIIYRIVDDNLPKFLENKA

SEQ ID NO: 31 - protein, 27 aa, synthetic construct
  REGION 1..27: note = Synthetic
FSAEDISTAIPHRIVQDNFPKFKENCH

SEQ ID NO: 32 - protein, 27 aa, synthetic construct
  REGION 1..27: note = Synthetic
YSDEEKSTAIAYRIVHENLPKFLDNIR

SEQ ID NO: 33 - protein, 27 aa, synthetic construct
  REGION 1..27: note = Synthetic
YSDEEKSTAIAYRLIHENLPKFIDNIK

SEQ ID NO: 34 - protein, 27 aa, synthetic construct
  REGION 1..27: note = Synthetic
YSDEEISTAIPFRIVNENFPKFLQNAE

SEQ ID NO: 35 - protein, 27 aa, synthetic construct
  REGION 1..27: note = Synthetic
FSKEKISSSACHRIVDDNAEIHFDNIR

SEQ ID NO: 36 - protein, 27 aa, synthetic construct
  REGION 1..27: note = Synthetic
FSKEDISSSICYRIVNENAEIFLQNIL

SEQ ID NO: 37 - protein, 27 aa, Clostridium sp. SCH47915.1
FSEDNISTAISFRIVNENSEIHLQNMR

SEQ ID NO: 38 - protein, 27 aa, Clostridium sp. SCH45297.1
FTKEAIATAIGYRVVHENAEIFLENMV

SEQ ID NO: 39 - protein, 26 aa, Eubacteriaceae bacterium
FADDKSTSICYRIVNENAWIFYQNYL

SEQ ID NO: 40 - protein, 27 aa, Firmicutes bacterium
FSSAGIATSICNRIVNENAEIFSDNKS

SEQ ID NO: 41 - protein, 27 aa, Clostridium sp. AM42-36
FSKEKISSAVGYRIVEENAEIFLQNQN

SEQ ID NO: 42 - protein, 27 aa, Lachnospira pectinoschiza
FSGEGGASSICHRIVNVNASIFYDNLK

SEQ ID NO: 43 - protein, 27 aa, Eubacterium sp.
FSKKPIHSSICHRTVDENTAIFYQNII

SEQ ID NO: 44 - protein, 27 aa, Coprococcus sp. AF19-8AC
FSDKAIASSISYRIIHENAKIYMDNLD

SEQ ID NO: 45 - protein, 50 aa, Eubacterium rectale
TQEGISFYNDICGKVNSFMNLYCQKNKENKNLYKLQKLHKQILCIADTSY

SEQ ID NO: 46 - protein, 63 aa, synthetic construct
  REGION 1..63: note = Synthetic
NQSGITKFNTIIGGKFVNGENTKRKGINEYINLYSQQINDKTLKKYKMSVLFKQILSDTESKS

SEQ ID NO: 47 - protein, 67 aa, synthetic construct
  REGION 1..67: note = Synthetic
TQTQIDLYNQLLGGISREAGTEKIKGLNEVLNLAIQKNDETAHIIASLPHRFIPLFKQILSDRNTLS

SEQ ID NO: 48 - protein, 52 aa, synthetic construct
  REGION 1..52: note = Synthetic
TQKGIDFYNAIIGGKKGLNEYINLYCQKHKKKKLPKLKPLHKQILSDRESLS

SEQ ID NO: 49 - protein, 59 aa, synthetic construct
  REGION 1..59: note = Synthetic
TQKGIDAYNAIIGGKTTEEGKKIKGLNEYINLYNQKHKDKLPKLKPLFKQILSDRESIS

SEQ ID NO: 50 - protein, 63 aa, synthetic construct
  REGION 1..63: note = Synthetic
TQDGIDYYNQIIGGVSEKAGDEKLRGINEFSNLYRQQHKEVAKDRIKMVPLYKQILSDRDTLS

SEQ ID NO: 51 - protein, 50 aa, synthetic construct
  REGION 1..50: note = Synthetic
SQEDISFYNDIVGKINKFMNLYCQKNKENKNLYKLRHLHKQILCIEESLY

SEQ ID NO: 52 - protein, 50 aa, synthetic construct
  REGION 1..50: note = Synthetic
TQKGIEFYNDICGKVNQHMNLYCQKNKENKNKYKMRKLHKQILSISESSF

SEQ ID NO: 53 - protein, 50 aa, Clostridium sp. SCH47915.1
TQPGIEYYNGICGKINEHMNQFCQKNRINKNDFRMKKLHKQILCKKSSYY

SEQ ID NO: 54 - protein, 50 aa, Clostridium sp. SCH45297.1
TQKAIEHYNEMCGVVNQHMKEYCQKEKKNWNLYRMKRLHKQILSNASTSF

SEQ ID NO: 55 - protein, 50 aa, Eubacteriaceae bacterium
NQKGIRFYNDICGIVNAHMNLYCQKYKKKAAKYRLKRMHKQILSIDESTF

SEQ ID NO: 56 - protein, 50 aa, Firmicutes bacterium
SQSGIDFYNMISGAVNKAVNEYCQKNGLNKNKYLLRKLRKQILSNSESTF

SEQ ID NO: 57 - protein, 51 aa, Clostridium sp. AM42-36
TQGGIDRYNEAIGAVNQYMNLLCQKNKALKPGQFKMKRLHKQILCKGTTSF

SEQ ID NO: 58 - protein, 50 aa, Lachnospira pectinoschiza
AQKGIDYYNQICGDINKHMNLYCQQNKFKANIFKMMKLQKQIMGISEKVF

SEQ ID NO: 59 - protein, 50 aa, Eubacterium sp.
TQQGIEFYNDICGIVNSHMNLYCQQTKEKSGQYRMRKLYKQILSISSTSY

SEQ ID NO: 60 - protein, 50 aa, Coprococcus sp. AF19-8AC
SQSGIDLYNNICGVINAHMNLYCQSKKCSRSKFKMQKLHKQILCKAETGF

SEQ ID NO: 61 - protein, 50 aa, Eubacterium rectale
IVSKFYESVSQKTYRDWETINTALEIHYNNILPGNGKSKADKVKKAVKND

SEQ ID NO: 62 - protein, 56 aa, synthetic construct
  REGION 1..56: note = Synthetic
FKNDKSLTDLSQQVFDDYSVIGTAVLEYITQQIAPKNLDNPSKKEQELIAKKTEKA

SEQ ID NO: 63 - protein, 51 aa, synthetic construct
  REGION 1..51: note = Synthetic
ISHKKLETISSALCDHWDTLRNALYERRISELTGKITKSAKEKVQRSLKHE

SEQ ID NO: 64 - protein, 50 aa, synthetic construct
  REGION 1..50: note = Synthetic
INDKQLTDISQKMFGDWSVIQDALKEYYPQKEKGKGKKKEEKIEKALKKD

SEQ ID NO: 65 - protein, 53 aa, synthetic construct
  REGION 1..53: note = Synthetic
IKNDLQLTDISQKMFGDWSIISRALDEYYVNPQKKKESKEKYEERKEKLLKKK

SEQ ID NO: 66 - protein, 50 aa, synthetic construct
  REGION 1..50: note = Synthetic
INQKKLTAISQELTGDWSVIEERMKEFAKEQEEDKKKSEEKKKEKELKSD

SEQ ID NO: 67 - protein, 50 aa, synthetic construct
  REGION 1..50: note = Synthetic
IVKKHFENISQKLYRDFEVINTALEIHYNDILPGNGKSKEDKVKKMVKND

SEQ ID NO: 68 - protein, 50 aa, synthetic construct
  REGION 1..50: note = Synthetic
ISSKNYESISNFMYGNWNTINDCLENYYEENIPGKGKKKEEKVKKAVKKD

SEQ ID NO: 69 - protein, 50 aa, Clostridium sp. SCH47915.1
ISSNKYEQISNALYGSWDTIRKCIKEEYMDALPGKGEKKEEKAEAAAKKE

SEQ ID NO: 70 - protein, 50 aa, Clostridium sp. SCH45297.1
ITAPYYEKISNYLCGSWNTIADCLTHYYEQQIAGKGARKDQKVKAAVKAD

SEQ ID NO: 71 - protein, 50 aa, Eubacteriaceae bacterium
VCEKNYENLSLFMCRNWSVLRDSIKAFYQENTTGSNAGKEKKIEKLMKED

SEQ ID NO: 72 - protein, 49 aa, Firmicutes bacterium
IAESAYEDVSIFMGYGWNGIKGCLEKKYEKEIAPGKAKDIKIKKLISQE

SEQ ID NO: 73 - protein, 50 aa, Clostridium sp. AM42-36
VVADAYSMISQFISKKWNLIEECLLDYYSDNLPGKGNAKENKVKKAVKEE

SEQ ID NO: 74 - protein, 50 aa, Lachnospira pectinoschiza
INARYYTNVSTYVYGGWGVIESAIERYLCNTIAGKGQSKVKKIENAKKDN

SEQ ID NO: 75 - protein, 50 aa, Eubacterium sp.
IASKNYSSISNFISGKWNTLDDCIRRYYEDNTVGNGDKKEKKVEEKVKKD

SEQ ID NO: 76 - protein, 50 aa, Coprococcus sp. AF19-8AC
ISSKAFENVSVYIDHKWDVIASSLYKYFSEIVKGNKDNREEKIQKEIKKV

SEQ ID NO: 77 - protein, 17 aa, Eubacterium rectale
SITEINELVSNYKLCSD

SEQ ID NO: 78 - protein, 27 aa, synthetic construct
  REGION 1..27: note = Synthetic
SLETIKLALEEFNKHRDIDKQCRFEEI

SEQ ID NO: 79 - protein, 16 aa, synthetic construct
  REGION 1..16: note = Synthetic
NLQEIISAAGKELSEA

SEQ ID NO: 80 - protein, 23 aa, synthetic construct
  REGION 1..23: note = Synthetic
SIADINKLLEEYESDEAKKIEEY

SEQ ID NO: 81 - protein, 23 aa, synthetic construct
  REGION 1..23: note = Synthetic
SIADIQEALDEYESVKAKNIEDY

SEQ ID NO: 82 - protein, 22 aa, synthetic construct
  REGION 1..22: note = Synthetic
SLEELDNILENCSDEEINIQEY

SEQ ID NO: 83 - protein, 17 aa, synthetic construct
  REGION 1..17: note = Synthetic
SIGEIDELVDNYNLCPD

SEQ ID NO: 84 - protein, 16 aa, synthetic construct
  REGION 1..16: note = Synthetic
SLAEIDKLVEKYNEEE

SEQ ID NO: 85 - protein, 17 aa, Clostridium sp. SCH47915.1
SIADIDKIISLYGSEMD

SEQ ID NO: 86 - protein, 17 aa, Clostridium sp. SCH45297.1
SLSEIEQLLKEYARAEE

SEQ ID NO: 87 - protein, 16 aa, Eubacteriaceae bacterium
SLQNINELINKYNSNS

SEQ ID NO: 88 - protein, 16 aa, Firmicutes bacterium
SIGEIDELFHIYGEEK

SEQ ID NO: 89 - protein, 19 aa, Clostridium sp. AM42-36
SVSQLNEVIEKYYVEKTGQ

SEQ ID NO: 90 - protein, 32 aa, Lachnospira pectinoschiza
SVKELDSIVAEYEPDYFNAPYIDDDDNAVKVF

SEQ ID NO: 91 - protein, 14 aa, Eubacterium sp.
SLDSIDKVVEMYGK

SEQ ID NO: 92 - protein, 19 aa, Coprococcus sp. AF19-8AC
SLGDLQRLVNSYYKIDSTC

SEQ ID NO: 93 - protein, 33 aa, Eubacterium rectale
PEIHLVESELKASELKNVLDVIMNAFHWCSVFM

SEQ ID NO: 94 - protein, 35 aa, synthetic construct
  REGION 1..35: note = Synthetic
GKKDLLQASAEDDVKAIKDLLDQTNNLLHKLKIFH

SEQ ID NO: 95 - protein, 26 aa, synthetic construct
  REGION 1..26: note = Synthetic
KQEEKEILKSQLDSLLGLYHLLDWFA

SEQ ID NO: 96 - protein, 33 aa, synthetic construct
  REGION 1..33: note = Synthetic
EEIKLIQNKEKVEEIKNLLDSIMDLQHFIKPLL

SEQ ID NO: 97 - protein, 33 aa, synthetic construct
  REGION 1..33: note = Synthetic
ENKKLAQDKANVEKIKNLLDAIKDLQHFIKPLL

SEQ ID NO: 98 - protein, 33 aa, synthetic construct
  REGION 1..33: note = Synthetic
EEQDLRENDEEVEHIKNYLDSLQNLLHRLKPLE

SEQ ID NO: 99 - protein, 33 aa, synthetic construct
  REGION 1..33: note = Synthetic
PEIHLVENELEIAELKEVIEVIMDIFHWCAKFK

SEQ ID NO: 100 - protein, 33 aa, synthetic construct
  REGION 1..33: note = Synthetic
EEIKLIENEEKAEEIKEVLDMYMNIFHWIKTFI

SEQ ID NO: 101 - protein, 31 aa, Eubacterium ventriosum
MNLIENETKSEEIKSKLDSIMEIMHWTKMFI

SEQ ID NO: 102 - protein, 33 aa, Eubacterium sp.
EHISLIESEEKADEMKKRLDMYMNMYHWAKAFI

SEQ ID NO: 103 - protein, 33 aa, Clostridium sp. SCH47915.1
SDIKLLQNKEKTTEIKTILDSFLHVYQWGQTFI

SEQ ID NO: 104 - protein, 33 aa, Clostridium sp. SCH45297.1
PEVNLIENEKYATEIKDVLDNYMELFHWMKWFY

SEQ ID NO: 105 - protein, 33 aa, Eubacteriaceae bacterium
EDISLIEDEESGEELKRVLDLIMSINHWIKMFI

SEQ ID NO: 106 - protein, 33 aa, Firmicutes bacterium
SSEKLTENDNKAAEIKNVLDYYFKIFHWIKTFI

SEQ ID NO: 107 - protein, 33 aa, Clostridium sp. AM42-36
EKHNLIEDDEKISEIKELLDMYMDVFHIIKVFR

SEQ ID NO: 108 - protein, 33 aa, Lachnospira pectinoschiza
SDDSLIENKESALRIKKQLDDIMSLYHWLQTFI

SEQ ID NO: 109 - protein, 33 aa, Eubacterium sp.
DSVKLIENDAKIEHIKCVLDMLLNTNRFLDTFT

SEQ ID NO: 110 - protein, 33 aa, Coprococcus sp. AF19-8AC
DKISLIQNEQIVMDIKTYLDKYMSIYHWMKSFV

SEQ ID NO: 111 - protein, 34 aa, Eubacterium rectale
KDNNFYAELEEIYDEIYPVISLYNLVRNYVTQKP

SEQ ID NO: 112 - protein, 34 aa, synthetic construct
  REGION 1..34: note = Synthetic
KDEHFYLVFEECYFELANIVPLYNKIRNYITQKP

SEQ ID NO: 113 - protein, 34 aa, synthetic construct
  REGION 1..34: note = Synthetic
VDPEFSARLTGIKLEMEPSLSFYNKARNYATKKP

SEQ ID NO: 114 - protein, 34 aa, synthetic construct
  REGION 1..34: note = Synthetic
KDENFYGEFEEIYEELDDITPLYNKVRNYVTQKP

SEQ ID NO: 115 - protein, 34 aa, synthetic construct
  REGION 1..34: note = Synthetic
KDERFYGEFTPLWDELDQITPLYNKVRNYLTQKP

SEQ ID NO: 116 - protein, 34 aa, synthetic construct
  REGION 1..34: note = Synthetic
KDTSFYSEFEEIYEELDEVILLYNKVRNYITQKP

SEQ ID NO: 117 - protein, 34 aa, synthetic construct
  REGION 1..34: note = Synthetic
KDNDFYAELEEINDEIHPIISLYNRVRNYVTQKP

SEQ ID NO: 118 - protein, 34 aa, synthetic construct
  REGION 1..34: note = Synthetic
KDVNFYSEIEDIYEEIEDIVPLYNRVRNYVTQKP

SEQ ID NO: 119 - protein, 34 aa, Eubacterium ventriosum
KDVNFYNEIEEIYDELQPLVTIYNRIRNYVTQKP

SEQ ID NO: 120 - protein, 34 aa, Eubacterium sp.
RDEMFYSDIDDIYNILENIVPLYNRVRNYVTQKP

SEQ ID NO: 121 - protein, 34 aa, Clostridium sp. SCH47915.1
KDSYFYSELEDVLEDFEGITTLYNHVRSYVTQKP

SEQ ID NO: 122 - protein, 34 aa, Clostridium sp. SCH45297.1
KEVNFYGELDDLYEEIRDIVPLYNKVRNYVTQKP

SEQ ID NO: 123 - protein, 34 aa, Eubacteriaceae bacterium
KDMAFYTEIEDIYYELEPLKSIYDKVRNYITQKP

SEQ ID NO: 124 - protein, 34 aa, Firmicutes bacterium
KDIVFYSGIEFAYEEIKDIVPLYNKVRNYVTQKP

SEQ ID NO: 125 - protein, 34 aa, Clostridium sp. AM42-36
FDETFYSEMDEIYQDMQEIVPLYNHVRNYVTQKP

SEQ ID NO: 126 - protein, 34 aa, Lachnospira pectinoschiza
KDNAFYAELEDICCELENVVTLYDRIRNYVTRKP

SEQ ID NO: 127 - protein, 34 aa, Eubacterium sp.
IDVGFYSEIDDLKEIIDGIDPLYNRVRNYVTRKP

SEQ ID NO: 128 - protein, 34 aa, Coprococcus sp. AF19-8AC
KDMEFYSELDELNEDMSEIVNLYNKVRNYVTQKP

SEQ ID NO: 129 - protein, 56 aa, Eubacterium rectale; identical to SEQ ID NO: 3

SEQ ID NO: 130 - protein, 61 aa, synthetic construct
  REGION 1..61: note = Synthetic
GANKFNDEINLLLKEKANDVHILSIDRGERHLAYYTLVDGKGNIIKQDTFNIIGNDRMKTN

SEQ ID NO: 131 - protein, 57 aa, synthetic construct
  REGION 1..57: note = Synthetic
NSPSKFNQRVNAYLKEHPETPIIGIDRGERNLIYITVIDSTGKILEQRSLNTIQQFD

SEQ ID NO: 132 - protein, 56 aa, synthetic construct
  REGION 1..56: note = Synthetic
GNSNINERVLKYIAKNDDMHIIGIDRGERNLLYVSVIDSKGNIVEQKSLNIINNTD

SEQ ID NO: 133 - protein, 64 aa, synthetic construct
  REGION 1..64: note = Synthetic
GNGNINQKVNDYLRSADDVHIIGIDRGERHLLYLVVIDSKGNIVEQFSLNEIVNEYNGNTYRTN

SEQ ID NO: 134 - protein, 57 aa, synthetic construct
  REGION 1..57: note = Synthetic
GNENINERVQEFLKNNPDVNIIGIDRGERHLIYLSLINQKGEILKQKTFNEVERNVD

SEQ ID NO: 135 - protein, 57 aa, synthetic construct
  REGION 1..57: note = Synthetic
NRRVNINERILQYIAQEKDLHIIGIDRGERNLIYVSVIDTDGNIVEQKSLNIINNVD

SEQ ID NO: 136 - protein, 56 aa, synthetic construct
  REGION 1..56: note = Synthetic
NRSNVNEMALKYIAKQDDMHIIGIDRGERNLIYVSVIDMHGNIVEQKSFNIVNGYD

SEQ ID NO: 137 - protein, 56 aa, Eubacterium ventriosum
GFSPINNIALKSIALKEDMHIIGIDRGERNLIYVSVIDTKGNIVEQRNFNIVNGID

SEQ ID NO: 138 - protein, 56 aa, Eubacterium sp.
ARNNVNDMAVKYIAQNDDIHVIGIDRGERNLIYISVIDSHGNIVKQKSYNILNNYD

SEQ ID NO: 139 - protein, 56 aa, Clostridium sp. SCH47915.1
SDIAVNERTLAYIAKKEDIHIIGIDRGERNLLYISVIDVHGNIREQRSFNIVNGYD

SEQ ID NO: 140 - protein, 56 aa, Clostridium sp. SCH45297.1
GKEALNSVAQRYIAHQNDMHVIGIDRGERNLIYVSVINMQGEIIEQKSFNVVNKYN

SEQ ID NO: 141 - protein, 56 aa, Eubacteriaceae bacterium
NYSPVNDIALKNIAENNDMHIIGIDRGERNLIYVSVIDLHGNIIEQKNFNIINGVN

SEQ ID NO: 142 - protein, 56 aa, Firmicutes bacterium
HTGNLNEMVIQYIAKQENMHVIGIDRGERNLIYVSVIDMNGKIKEQKSFNIVNSYN

SEQ ID NO: 143 - protein, 65 aa, Clostridium sp. AM42-36
KGNNVNAIAQQYIAEQEDLHVIGIDRGERNLIYVSVIDMYGRILEQKSFNLVEQVSSQGTKRYYD

SEQ ID NO: 144 - protein, 55 aa, Lachnospira pectinoschiza
DENVNSKIIEYIAKQDNMNVIGIDRGERNLIYISVIDNKGNIIEQKSFNLVNNYD

SEQ ID NO: 145 - protein, 58 aa, Eubacterium sp.
GASDKQLNEQVLEYISKQDDMHIIGIDRGERNLVYVSVIDMKGRIVEQKSYNVVNSYS

SEQ ID NO: 146 - protein, 66 aa, Coprococcus sp. AF19-8AC
GRININEKVLKYIAENDELHVIGIDRGERNLLYVSVINKKGKIVEQKSFNMIESYETVTNIVRRYN

SEQ ID NO: 147 - protein, 17 aa, Eubacterium rectale
YQIKLKQQEGARQIARK

SEQ ID NO: 148 - protein, 17 aa, synthetic construct
  REGION 1..17: note = Synthetic
YHDKLAAIEKDRDSARK

SEQ ID NO: 149 - protein, 17 aa, synthetic construct
  REGION 1..17: note = Synthetic
YQKKLDNREKERVAARQ

SEQ ID NO: 150 - protein, 17 aa, synthetic construct
  REGION 1..17: note = Synthetic
YHAKLDQREKERDEARK

SEQ ID NO: 151 - protein, 17 aa, synthetic construct
  REGION 1..17: note = Synthetic
YHDLLDKREKERLKARQ

SEQ ID NO: 152 - protein, 17 aa, synthetic construct
  REGION 1..17: note = Synthetic
YQAKLEQREKERDEARK

SEQ ID NO: 153 - protein, 17 aa, synthetic construct
  REGION 1..17: note = Synthetic
YQIKLKQQEIMRQIARQ

SEQ ID NO: 154 - protein, 17 aa, synthetic construct
  REGION 1..17: note = Synthetic
YQEKLKQREKDRDEARK

SEQ ID NO: 155 - protein, 17 aa, Eubacterium ventriosum
YKEKLKQKELDRDNARK

SEQ ID NO: 156 - protein, 17 aa, Eubacterium sp.
YKKKLVEKEKTREYARK

SEQ ID NO: 157 - protein, 17 aa, Clostridium sp. SCH47915.1
YQQKLKDREKSRDAARK

SEQ ID NO: 158 - protein, 17 aa, Clostridium sp. SCH45297.1
YKEKLKEREQNRDEARK

SEQ ID NO: 159 - protein, 17 aa, Eubacteriaceae bacterium
YKEKLKQRESERDSARK

SEQ ID NO: 160 - protein, 17 aa, Firmicutes bacterium
YQEKLRGREKDRLNARK

SEQ ID NO: 161 - protein, 17 aa, Clostridium sp. AM42-36
YKEKLQNREEERDKARK

SEQ ID NO: 162 - protein, 17 aa, Lachnospira pectinoschiza
YKNKLKNMEKTRDNARK

SEQ ID NO: 163 - protein, 17 aa, Eubacterium sp.
YQKKLVERERTRDEARK

SEQ ID NO: 164 - protein, 17 aa, Coprococcus sp. AF19-8AC
YKDKLVNKESARTDARK

SEQ ID NO: 165 - protein, 32 aa, Eubacterium rectale
EWKEIGKIKEIKEGYLSLVIHEISKMVIKYNA

SEQ ID NO: 166 - protein, 32 aa, synthetic construct
  REGION 1..32: note = Synthetic
DWKKINNIKEMKEGYLSQVVHEIAKLVIEYNA

SEQ ID NO: 167 - protein, 32 aa, synthetic construct
  REGION 1..32: note = Synthetic
AWSVVGTIKDLKQGYLSQVIHEIVDLMIHYQA

SEQ ID NO: 168 - protein, 32 aa, synthetic construct
  REGION 1..32: note = Synthetic
NWKTIENIKELKEGYLSQVIHEIAELMIKYNA

SEQ ID NO: 169 - protein, 32 aa, synthetic construct
  REGION 1..32: note = Synthetic
SWQTIENIKELKEGYLSQVIHKISELMIKYNA

SEQ ID NO: 170 - protein, 32 aa, synthetic construct
  REGION 1..32: note = Synthetic
NWKTIGKIKELKEGYLSAVIHEITKMMIENNA

SEQ ID NO: 171 - protein, 32 aa, synthetic construct
  REGION 1..32: note = Synthetic
EWKEIVKIKEIKEGYLSQVIHEIAELVIKYNA

SEQ ID NO: 172 - protein, 32 aa, synthetic construct
  REGION 1..32: note = Synthetic
NWKEIGKIKELKEGYLSLVIHEIAKLVIKYNA

SEQ ID NO: 173 - protein, 32 aa, Eubacterium ventriosum
NWKEIGKIKDLKEGYLSLVVHEIAKLVVKYNA

SEQ ID NO: 174 - protein, 32 aa, Eubacterium sp.
NWKSIGNIKELKEGYISGVVHEIAMLMVEYNA

SEQ ID NO: 175 - protein, 32 aa, Clostridium sp. SCH47915.1
NWEEIEKIKELKEGYLSMVIHYIARLVVKYNA

SEQ ID NO: 176 - protein, 32 aa, Clostridium sp. SCH45297.1
NWKEIGQIKDLKEGYLSGVIHEIAKMMIKYHA

SEQ ID NO: 177 - protein, 32 aa, Eubacteriaceae bacterium
NWKQIGKIKDIKEGYLSLVIHEITSLVLKYNA

SEQ ID NO: 178 - protein, 32 aa, Firmicutes bacterium
NWKQIANIKEMKEGYLSLVIHEITEMMMKYNA

SEQ ID NO: 179 - protein, 32 aa, Clostridium sp. AM42-36
SWKTIGKIKELKEGYLSSVIHEIAQMVVKYNA

SEQ ID NO: 180 - protein, 32 aa, Lachnospira pectinoschiza
NWQEIGKIKDVKSGYLSGVISKIARMVIDYNA

SEQ ID NO: 181 - protein, 32 aa, Eubacterium sp.
SWKEVGRIKDLKDGYLSLVVHEIADMVIKYNA

SEQ ID NO: 182 - protein, 32 aa, Coprococcus sp. AF19-8AC
NWKEIGKIKEIKEGYLSQVIHEISKMVLKYNA

SEQ ID NO: 183 - protein, 35 aa, Eubacterium rectale
IIAMEDLSYGFKKGRFKVERQVYQKFETMLINKLN

SEQ ID NO: 184 - protein, 35 aa, synthetic construct
  REGION 1..35: note = Synthetic
IVVFEDLNFGFKRGRFKVEKQVYQKLEKMLIEKLN

SEQ ID NO: 185 - protein, 36 aa, synthetic construct
  REGION 1..36: note = Synthetic
VVVLENLNFGFKSKRTGIAEKAVYQQFEKMLIDKLN

SEQ ID NO: 186 - protein, 35 aa, synthetic construct
  REGION 1..35: note = Synthetic
IVVMEDLNFGFKRGRFKVEKQVYQKFEKMLIDKLN

SEQ ID NO: 187 - protein, 35 aa, synthetic construct
  REGION 1..35: note = Synthetic
IVVLEDLNFGFKRGRQKVEKQVYQKFEKMLIDKLN

SEQ ID NO: 188 - protein, 35 aa, synthetic construct
  REGION 1..35: note = Synthetic
IIVMEDLNFGFKRGRFKVERQVYQKFEKMLIDKLN

SEQ ID NO: 189 - protein, 35 aa, synthetic construct
  REGION 1..35: note = Synthetic
IIVMEDLNSRFKEKRSKIERQVYQQFETMLINKLN

SEQ ID NO: 190 - protein, 35 aa, synthetic construct
  REGION 1..35: note = Synthetic
IIAMEDLNYGFKRGRFKVERQVYQKFETMLINKLN

SEQ ID NO: 191 - protein, 35 aa, Eubacterium ventriosum
IITMEDLNQGFKRGRFKVERQVYQKFETMLINKLN

SEQ ID NO: 192 - protein, 35 aa, Eubacterium sp.
IIAMEDLNYGFKRGRFKVERQVYQKFESMLINKLN

SEQ ID NO: 193 - protein, 35 aa, Clostridium sp. SCH47915.1
VVAMEDLNYGFKTGRFKVERQVYQKFETMLIEKLH

SEQ ID NO: 194 - protein, 35 aa, Clostridium sp. SCH45297.1
IVAMEDLNYGFKRGRFKVERQVYQKFENMLIQKLN

SEQ ID NO: 195 - protein, 17 aa, Eubacteriaceae bacterium
YKEKLKQKELDRDNARK

SEQ ID NO: 196 - protein, 17 aa, Firmicutes bacterium
YKKKLVEKEKTREYARK

SEQ ID NO: 197 - protein, 17 aa, Clostridium sp. AM42-36
YQQKLKDREKSRDAARK

SEQ ID NO: 198 - protein, 17 aa, Lachnospira pectinoschiza
YKEKLKEREQNRDEARK

SEQ ID NO: 199 - protein, 17 aa, Eubacterium sp.
YKEKLKQRESERDSARK

SEQ ID NO: 200 - protein, 17 aa, Coprococcus sp. AF19-8AC
YQEKLRGREKDRLNARK

SEQ ID NO: 201 - protein, 17 aa, Eubacterium rectale
YKEKLQNREEERDKARK

SEQ ID NO: 202 - protein, 17 aa, synthetic construct
  REGION 1..17: note = Synthetic
YKNKLKNMEKTRDNARK

SEQ ID NO: 203 - protein, 17 aa, synthetic construct
  REGION 1..17: note = Synthetic
YQKKLVERERTRDEARK

SEQ ID NO: 204 - protein, 17 aa, synthetic construct
  REGION 1..17: note = Synthetic
YKDKLVNKESARTDARK

SEQ ID NO: 205 - protein, 32 aa, synthetic construct; identical to SEQ ID NO: 165
  REGION 1..32: note = Synthetic

SEQ ID NO: 206 - protein, 32 aa, synthetic construct; identical to SEQ ID NO: 166
  REGION 1..32: note = Synthetic

SEQ ID NO: 207 - protein, 32 aa, synthetic construct; identical to SEQ ID NO: 167
  REGION 1..32: note = Synthetic

SEQ ID NO: 208 - protein, 32 aa, synthetic construct; identical to SEQ ID NO: 168
  REGION 1..32: note = Synthetic

SEQ ID NO: 209 - protein, 32 aa, Eubacterium ventriosum; identical to SEQ ID NO: 169

SEQ ID NO: 210 - protein, 32 aa, Eubacterium sp.; identical to SEQ ID NO: 170

SEQ ID NO: 211 - protein, 32 aa, Clostridium sp. SCH47915.1; identical to SEQ ID NO: 171

SEQ ID NO: 212 - protein, 32 aa, Clostridium sp. SCH45297.1; identical to SEQ ID NO: 172

SEQ ID NO: 213 - protein, 32 aa, Eubacteriaceae bacterium; identical to SEQ ID NO: 173

SEQ ID NO: 214 - protein, 32 aa, Firmicutes bacterium; identical to SEQ ID NO: 174

SEQ ID NO: 215 - protein, 32 aa, Clostridium sp. AM42-36; identical to SEQ ID NO: 175

SEQ ID NO: 216 - protein, 32 aa, Lachnospira pectinoschiza; identical to SEQ ID NO: 176

SEQ ID NO: 217 - protein, 32 aa, Eubacterium sp.; identical to SEQ ID NO: 177

SEQ ID NO: 218 - protein, 32 aa, Coprococcus sp. AF19-8AC; identical to SEQ ID NO: 178

SEQ ID NO: 219 - protein, 32 aa, Eubacterium rectale; identical to SEQ ID NO: 179

SEQ ID NO: 220 - protein, 32 aa, synthetic construct; identical to SEQ ID NO: 180
  REGION 1..32: note = Synthetic

SEQ ID NO: 221 - protein, 32 aa, synthetic construct; identical to SEQ ID NO: 181
  REGION 1..32: note = Synthetic

SEQ ID NO: 222 - protein, 32 aa, synthetic construct; identical to SEQ ID NO: 182
  REGION 1..32: note = Synthetic

SEQ ID NO: 223 - protein, 35 aa, synthetic construct; identical to SEQ ID NO: 183
  REGION 1..35: note = Synthetic

SEQ ID NO: 224 - protein, 35 aa, synthetic construct; identical to SEQ ID NO: 184
  REGION 1..35: note = Synthetic

SEQ ID NO: 225 - protein, 36 aa, synthetic construct; identical to SEQ ID NO: 185
  REGION 1..36: note = Synthetic

SEQ ID NO: 226 - protein, 35 aa, synthetic construct; identical to SEQ ID NO: 186
  REGION 1..35: note = Synthetic

SEQ ID NO: 227 - protein, 35 aa, Eubacterium ventriosum; identical to SEQ ID NO: 187

SEQ ID NO: 228 - protein, 35 aa, Eubacterium sp.; identical to SEQ ID NO: 188

SEQ ID NO: 229 - protein, 35 aa, Clostridium sp. SCH47915.1; identical to SEQ ID NO: 189

SEQ ID NO: 230 - protein, 35 aa, Clostridium sp. SCH45297.1; identical to SEQ ID NO: 190

SEQ ID NO: 231 - protein, 35 aa, Eubacteriaceae bacterium; identical to SEQ ID NO: 191

SEQ ID NO: 232 - protein, 35 aa, Firmicutes bacterium; identical to SEQ ID NO: 192

SEQ ID NO: 233 - protein, 35 aa, Clostridium sp. AM42-36; identical to SEQ ID NO: 193

SEQ ID NO: 234 - protein, 35 aa, Lachnospira pectinoschiza; identical to SEQ ID NO: 194

SEQ ID NO: 235 - protein, 35 aa, Eubacterium sp.
IIAMEDLNMGFKRGRFKVERQVYQKFENMLISKLN

SEQ ID NO: 236 - protein, 35 aa, Coprococcus sp. AF19-8AC
IIAMEDLNYGFKRGRFKVERQVYQKFETMLISKLN

SEQ ID NO: 237 - protein, 35 aa, Eubacterium rectale; identical to SEQ ID NO: 236

SEQ ID NO: 238 - protein, 35 aa, synthetic construct
  REGION 1..35: note = Synthetic
IIVMEDLNKGFKRGRFKVERQVYQKFENMLISKLN

SEQ ID NO: 239 - protein, 35 aa, synthetic construct
  REGION 1..35: note = Synthetic
IIAMEDLNYGFKRGRFKIERQVYQKFESMLISKLS

SEQ ID NO: 240 - protein, 35 aa, synthetic construct
  REGION 1..35: note = Synthetic
IIVMEDLNYGFKRGRFRVERQVYQKFENMLISKLA

SEQ ID NO: 241 - protein, 18 aa, synthetic construct
  REGION 1..18: note = Synthetic
IPDKLKNVGHQCGCIFYV

SEQ ID NO: 242 - protein, 18 aa, synthetic construct
  REGION 1..18: note = Synthetic
PFETFKKMGKQTGIIYYV

SEQ ID NO: 243 - protein, 18 aa, synthetic construct
  REGION 1..18: note = Synthetic
QFTSFAKMGTQSGFLFYV

SEQ ID NO: 244 - protein, 18 aa, synthetic construct
  REGION 1..18: note = Synthetic
KFESFKKLGKQCGFIFYV

SEQ ID NO: 245 - protein, 18 aa, Eubacterium ventriosum
KFESFKKLGKQSGFLFYV

SEQ ID NO: 246 - protein, 18 aa, Eubacterium sp.
KFESFQKLGKQSGFIFYI

SEQ ID NO: 247 - protein, 18 aa, Clostridium sp. SCH47915.1
IPEKLKNVGHQCGCILYV

SEQ ID NO: 248 - protein, 18 aa, Clostridium sp. SCH45297.1
IPESLKNLGRQCGIIFYV

SEQ ID NO: 249 - protein, 18 aa, Eubacteriaceae bacterium
IPESLKVLGRQCGYIFYV

SEQ ID NO: 250 - protein, 18 aa, Firmicutes bacterium
VPDNIKNLGKQCGVIFYV

SEQ ID NO: 251 - protein, 18 aa, Clostridium sp. AM42-36
IPESLKKVGKQCGFIFYV

SEQ ID NO: 252 - protein, 18 aa, Lachnospira pectinoschiza
IPDSVKKLGRQCGMIFYV

SEQ ID NO: 253 - protein, 18 aa, Eubacterium sp.
IPKSLKELGRQCGYIFYV

SEQ ID NO: 254 - protein, 18 aa, Coprococcus sp. AF19-8AC
VPASLDRLGRQCGFIFYV

SEQ ID NO: 255 - protein, 18 aa, Eubacterium rectale
VPDNIKNVGRQCGIIFYV

SEQ ID NO: 256 - protein, 18 aa, synthetic construct
  REGION 1..18: note = Synthetic
IPKSIKNVGKQCGCIFYV

SEQ ID NO: 257 - protein, 18 aa, synthetic construct
  REGION 1..18: note = Synthetic
VPKDVKKVGRQCGIIFYV

SEQ ID NO: 258 - protein, 18 aa, synthetic construct
  REGION 1..18: note = Synthetic
IPDSLEKLGSQCGIIFYV

SEQ ID NO: 259 - protein, 35 aa, synthetic construct
  REGION 1..35: note = Synthetic
PAAYTSKIDPTTGFVNIFKFKDLTVDAKREFIKKF

SEQ ID NO: 260 - protein, 35 aa, synthetic construct
  REGION 1..35: note = Synthetic
PAGFTSKICPVTGFVNQLYPKYESVSKSQEFFSKF

SEQ ID NO: 261 - protein, 36 aa, synthetic construct
  REGION 1..36: note = Synthetic
PAPYTSKIDPLTGFVDPFVWKTIKNHESRKHFLEGF

SEQ ID NO: 262 - protein, 35 aa, synthetic construct
  REGION 1..35: note = Synthetic
PAWYTSKIDPTTGFVNLFNFKYENVEKAKDFFGKF

SEQ ID NO: 263 - protein, 35 aa, Eubacterium ventriosum
PAWNTSKIDPVTGFVNLFDPRYENVEKAKAFFGKF

SEQ ID NO: 264 - protein, 36 aa, Eubacterium sp.
PAAYTSKIDPKSGFVDLFNLNDLTNKEKKKDFFMKL

SEQ ID NO: 265 - protein, 36 aa, Clostridium sp. SCH47915.1
PAAYTSKIDPTTGFVNIFKFKDISSEDAKREFIKRF

SEQ ID NO: 266 - protein, 35 aa, Clostridium sp. SCH45297.1
PAAYTSKIDPTTGFVDIFNFKELTDEARRDFISKF

SEQ ID NO: 267 - protein, 32 aa, Eubacteriaceae bacterium
PVAYTSKIDPTTGFVAIFNYKGMTDKDFVTSF

SEQ ID NO: 268 - protein, 36 aa, Firmicutes bacterium
PAAFTSKIDPSTGFISAFNFKSISTNASRKQFFMQF

SEQ ID NO: 269 - protein, 36 aa, Clostridium sp. AM42-36
PAGYTSKIDPTTGFVNLFSFKNLTNRESRQDFVGEF

SEQ ID NO: 270 - protein, 36 aa, Lachnospira pectinoschiza
PAAFTSKIDPATGFVDIFNHKAYTTDQAKREFILSF

SEQ ID NO: 271 - protein, 32 aa, Eubacterium sp.
PAAYTSKIDPTTGFVSVFNYKEMDDEKFVTSF

SEQ ID NO: 272 - protein, 36 aa, Coprococcus sp. AF19-8AC
PAAYTSKIDPTTGFVDLFNHSELIKAGKRRDNLSKF

SEQ ID NO: 273 - protein, 36 aa, Eubacterium rectale
PAAYTSKIDPTTGFINAFKRDVVSTNDAKENFLMKF

SEQ ID NO: 274 - protein, 42 aa, synthetic construct
  REGION 1..42: note = Synthetic
PAAYTSKIDPATGFINIFDFKKYSGSGINAKVKDKKEFLMSM

SEQ ID NO: 275 - protein, 42 aa, synthetic construct
  REGION 1..42: note = Synthetic
PPAYTSKIDPATGFVDLFKFKSGEKEGTARADNDRKEFLSKF

SEQ ID NO: 276 - protein, 36 aa, synthetic construct
  REGION 1..36: note = Synthetic
PAAYTSKIDPLTGFVNVFNFREYSNFETKLDFVRSL

SEQ ID NO: 277 - protein, 28 aa, synthetic construct
  REGION 1..28: note = Synthetic
LFCFTFDYNNFITQNTVMSKSSWSVYTY

SEQ ID NO: 278 - protein, 25 aa, synthetic construct
  REGION 1..25: note = Synthetic
YFEFSFDYKNFGDKAAKGKWTIASF

SEQ ID NO: 279 - protein, 45 aa, synthetic construct
  REGION 1..45: note = Synthetic
DFILHFKMNRNLSFQRGLPGFMPAWDIVFEKNETQFDAKGTPFIA

SEQ ID NO: 280 - protein, 27 aa, synthetic construct
  REGION 1..27: note = Synthetic
YFEFAFDYNNFTHKAEGARTKWTVCTY

SEQ ID NO: 281 - protein, 27 aa, Eubacterium ventriosum
YFEFEFDYNNFTKKAEGTRTKWTVCTY

SEQ ID NO: 282 - protein, 26 aa, Eubacterium sp.
NFEFEFDYDKFRKQTDYQNKWTVSTN

SEQ ID NO: 283 - protein, 28 aa, Clostridium sp. SCH47915.1
LFAFEFDYDNFETQNEVMARSKWSVYTY

SEQ ID NO: 284 - protein, 28 aa, Clostridium sp. SCH45297.1
LFAFTFDYNNFITHNTTLAKNKWTIYTN

SEQ ID NO: 285 - protein, 28 aa, Eubacteriaceae bacterium
LFAFEFDYENFVTHKVEMARNKWTVYTY

SEQ ID NO: 286 - protein, 28 aa, Firmicutes bacterium
MFSFGFDYNNFDTYNITMGKTQWTVYTN

SEQ ID NO: 287 - protein, 28 aa, Clostridium sp. AM42-36
MFEFSFDYNNYIKKGTMLASTKWKVYTN

SEQ ID NO: 288 - protein, 28 aa, Lachnospira pectinoschiza
LFRFTFDYANFATHNVTLARNNWTIYTN

SEQ ID NO: 289 - protein, 28 aa, Eubacterium sp.
KFALKFDYTNFITHNVKLAKNEWTIYSN

SEQ ID NO: 290 - protein, 28 aa, Coprococcus sp. AF19-8AC
MFCYAFDYKNFVTHNTDIYQNSWEIYTN

SEQ ID NO: 291 - protein, 28 aa, Eubacterium rectale
LFKFSFDYKNFATHKLTLAKTKWDVYTN

SEQ ID NO: 292 - protein, 28 aa, synthetic construct
  REGION 1..28: note = Synthetic
LFAFSFDYNNFKTYNVSSPVNEWTAYTY

SEQ ID NO: 293 - protein, 28 aa, synthetic construct
  REGION 1..28: note = Synthetic
MFAFTFDYDNFAMHNTVIAKKKWTAYTF

SEQ ID NO: 294 - protein, 28 aa, synthetic construct
  REGION 1..28: note = Synthetic
LFSISFDYDNFKTHNTTLAKTKWVIYLR

SEQ ID NO: 295 - protein, 43 aa, synthetic construct
  REGION 1..43: note = Synthetic
GVRIKRRFVNGRFSNESDTIDITKDMEKTLEMTDINWRDGHDL

SEQ ID NO: 296 - protein, 44 aa, synthetic construct
  REGION 1..44: note = Synthetic
GSRLINFRNSDKNHNWDTREVYPTKELEKLLKDYSIEYGHGECI

SEQ ID NO: 297 - protein, 43 aa, synthetic construct
  REGION 1..43: note = Synthetic
GKRIVPVIENHRFTGRYRDLYPANELIALLEEKGIVFRDGSNI

SEQ ID NO: 298 - protein, 40 aa, synthetic construct
  REGION 1..40: note = Synthetic
GERIKTKFKNGRWDTEEIDLTEEMKKLFEKYGIEYKGHDL

SEQ ID NO: 299 - protein, 42 aa, Eubacterium ventriosum
GERIYTFRNPEKNNQWDNEEIDLTKELKSLFEKYGIDIKSDL

SEQ ID NO: 300 - protein, 39 aa, Eubacterium sp.
GKRIVKDKDEKGMNDREPTEDIKQIFEQKEIKIHEGEDL

SEQ ID NO: 301 - protein, 43 aa, Clostridium sp. SCH47915.1
GVRIKRRFRNRRFSNEEDIIDITEEIEKTLEMTDINWRDSHDI

SEQ ID NO: 302 - protein, 43 aa, Clostridium sp. SCH45297.1
GTRIKKEFVNGRWTDKTEEIDLTEEMKKLLEDTEIEYADGHDL

SEQ ID NO: 303 - protein, 42 aa, Eubacteriaceae bacterium
GERIKRKFKNGLWDTAEKVDLTYQMRSILEKYEIEYNKGQDI

SEQ ID NO: 304 - protein, 43 aa, Firmicutes bacterium
GERLQSEFNNARRTGKTKSINLTETIKLLLKDNEINYADGHDI

SEQ ID NO: 305 - protein, 43 aa, Clostridium sp. AM42-36
GTRLKRIVVNGKYTSQSMEVELTDAMEKMLQRAGIEYHDGKDL

SEQ ID NO: 306 - protein, 43 aa, Lachnospira pectinoschiza
GTRTQKEFVNRRVRDKKEVFDPTEKMLKLLELEGVEYQSGANL

SEQ ID NO: 307 - protein, 42 aa, Eubacterium sp.
GTRKIRKYRNDKWNSPDNVNLTNEIIKLMEQYNIQYDNEQDI

SEQ ID NO: 308 - protein, 43 aa, Coprococcus sp. AF19-8AC
KERLRKIFGNGRPTGKTEKIELTQMMKEVLTGAGVEYKDGHNL

SEQ ID NO: 309 - protein, 41 aa, Eubacterium rectale
GTRIQNMKVEGHWLSMEVELTTKMKELLDDSHIPYEEGQNI

SEQ ID NO: 310 - protein, 42 aa, synthetic construct
  REGION 1..42: note = Synthetic
GERIKKLYKDGRWLRSEVLNLTENLIKLMEQYNIEYKDGHDI

SEQ ID NO: 311 - protein, 43 aa, synthetic construct
  REGION 1..43: note = Synthetic
GSRIQKVYENGRYTSNTREIELSDKMKRLLNENNIEYGDGHNL

SEQ ID NO: 312 - protein, 41 aa, synthetic construct
  REGION 1..41: note = Synthetic
GERIKKEHTSYGWKDDVWNVESRIKDLFDSSHMKYDDGHNL

SEQ ID NO: 313 - protein, 14 aa, synthetic construct
  REGION 1..14: note = Synthetic
IVQHIFEIFRLTVQ

SEQ ID NO: 314 - protein, 14 aa, synthetic construct
  REGION 1..14: note = Synthetic
FFAKLTSVLNTILQ

SEQ ID NO: 315 - protein, 14 aa, synthetic construct
  REGION 1..14: note = Synthetic
AIDTMVALIRSVLQ

SEQ ID NO: 316 - protein, 14 aa, synthetic construct
  REGION 1..14: note = Synthetic
FFKELLYLFKLTLQ

SEQ ID NO: 317 - protein, 14 aa, Eubacterium ventriosum
FFKELMYLLKLTLQ

SEQ ID NO: 318 - protein, 14 aa, Eubacterium sp.
FASELLYNFKNTLQ

SEQ ID NO: 319 - protein, 14 aa, Clostridium sp. SCH47915.1
IVQHIFEIFKLTVQ

SEQ ID NO: 320 - protein, 14 aa, Clostridium sp. SCH45297.1
IIKEIFDIFRLTVQ

SEQ ID NO: 321 - protein, 14 aa, Eubacteriaceae bacterium
ICKEIKYLVKDIVQ

SEQ ID NO: 322 - protein, 14 aa, Firmicutes bacterium
FFAQLLYLYKLTVQ

SEQ ID NO: 323 - protein, 14 aa, Clostridium sp. AM42-36
IEAEIIDIFRLTVQ

SEQ ID NO: 324 - protein, 14 aa, Lachnospira pectinoschiza
LFHELQRIVRFTVQ

SEQ ID NO: 325 - protein, 14 aa, Eubacterium sp.
FCKEMKKLVKYIVQ

SEQ ID NO: 326 - protein, 14 aa, Coprococcus sp. AF19-8AC
CIKQVLDIFLYSIQ

SEQ ID NO: 327 - protein, 14 aa, Eubacterium rectale
IVNGILEIFWLTVQ

SEQ ID NO: 328 - protein, 14 aa, synthetic construct
  REGION 1..14: note = Synthetic
FICSLFEELKYTVQ

SEQ ID NO: 329 - protein, 14 aa, synthetic construct
  REGION 1..14: note = Synthetic
VINEIFKIFRLTVQ

SEQ ID NO: 330 - protein, 14 aa, synthetic construct
  REGION 1..14: note = Synthetic
LINELIEIIRLTVQ

SEQ ID NO: 331 - protein, 39 aa, synthetic construct
  REGION 1..39: note = Synthetic
MRNSLSELEDRDYDRLISPVLNENNIFYDSAKAGDALPK

SEQ ID NO: 332 - protein, 36 aa, synthetic construct
  REGION 1..36: note = Synthetic
MRNSKTGTELDYLISPVADVNGNFFDSRQAPKNMPQ

SEQ ID NO: 333 - protein, 36 aa, synthetic construct
  REGION 1..36: note = Synthetic
MRNSNAATGEDYINSPVRDLNGVCFDSRFQNPEWPM

SEQ ID NO: 334 - protein, 36 aa, synthetic construct
  REGION 1..36: note = Synthetic
MRNSKTETEYDYIISPVLNEEGEFFDSRKADKSLPK

SEQ ID NO: 335 - protein, 36 aa, Eubacterium ventriosum
MRNSNTGTDIDYLISPVANENGNFFDSRKADDSLPQ

SEQ ID NO: 336 - protein, 36 aa, Eubacterium sp.
MRNSNADTGEDYIISPVKNDDGQFFDSREQDKKLPI

SEQ ID NO: 337 - protein, 39 aa, Clostridium sp. SCH47915.1
MRNSLSELEDREYDRLISPILNENNKFFDSDKADDALPK

SEQ ID NO: 338 - protein, 39 aa, Clostridium sp. SCH45297.1
MRNSKSENEDREYDRIISPVLNEEGEFFDSDKYDKDLPK

SEQ ID NO: 339 - protein, 39 aa, Eubacteriaceae bacterium
MRNSLPDNAVEDYDAIISPVINNNGEFFDSTRGDEDKPL

SEQ ID NO: 340 - protein, 49 aa, Firmicutes bacterium
MRNSYTEAEEQEKGISYDKIISPVINDEGDFFDSDNYKESDDKECKMPK

SEQ ID NO: 341 - protein, 39 aa, Clostridium sp. AM42-36
MRNSRSESEDREYDRLISPVLNDKGEFFDTATADKTLPQ

SEQ ID NO: 342 - protein, 46 aa, Lachnospira pectinoschiza
LRNSKNEENDVDYDHVISPVLNEEGKFFDSSKYENKEEKKESLLPV

SEQ ID NO: 343 - protein, 39 aa, Eubacterium sp.
MRNSLPDNDSIEYDEIISPVLNESGEFYNSEEKNKKLPL

SEQ ID NO: 344 - protein, 51 aa, Coprococcus sp. AF19-8AC
LRNSKGENEDSKESDYDRIISPVLNQENEFFDSVVYADKYKKDEKLADKPI